European Patent Specification EP 4 031 569 B1, published August 20, 2025. Title: ANTI-STEM CELL FACTOR ANTIBODIES AND METHODS OF USE THEREOF. Applicant: Opsidio, LLC. The sequence listing filed with the application follows.

SEQUENCE LISTING (50 sequences)

SEQ ID NO: 1 - protein, 5 aa, Mus musculus
SYWMN

SEQ ID NO: 2 - protein, 17 aa, Mus musculus
QIYPGDGDTHYNGKFKG

SEQ ID NO: 3 - protein, 7 aa, Mus musculus
SNWVGSY

SEQ ID NO: 4 - protein, 16 aa, Mus musculus
KSSQSLLESDGKTYLN

SEQ ID NO: 5 - protein, 7 aa, Mus musculus
LVSRLDS

SEQ ID NO: 6 - protein, 9 aa, Mus musculus
WQGTHLPQT

SEQ ID NO: 7 - protein, 116 aa, Mus musculus
QVQLQQSGAELVRPGSSVKISCKSSGYAFSSYWMNWVKQRPGQGLEWIGQIYPGDGDTHYNGKFKGKATLTADKSSSTAYMQLSRLTSEDSAVYFCSSSNWVGSYWGQGTLVTVSA

SEQ ID NO: 8 - protein, 116 aa, Artificial Sequence
  Humanized 5H10 Heavy chain variable region VH1
QVQLVQSGAELKKPGSSVKISCKSSGYAFSSYWMNWVKQRPGQGLEWIGQIYPGDGDTHYNGKFKGKATLTADKSTSTAYMELSSLTSEDSAVYFCSSSNWVGSYWGQGTLVTVSS

SEQ ID NO: 9 - protein, 116 aa, Artificial Sequence
  Humanized 5H10 Heavy chain variable region VH2
QVQLVQSGAEVKKPGSSVKISCKSSGYAFSSYWMNWVKQRPGQGLEWIGQIYPGDGDTHYNGKFKGKATLTADKSTSTAYMELSSLRSEDTAVYFCSSSNWVGSYWGQGTLVTVSS

SEQ ID NO: 10 - protein, 116 aa, Artificial Sequence
  Humanized 5H10 Heavy chain variable region VH3
QVQLVQSGAEVKKPGSSVKVSCKSSGYAFSSYWMNWVRQRPGQGLEWIGQIYPGDGDTHYNGKFKGKATLTADKSTSTAYMELSSLRSEDTAVYFCSSSNWVGSYWGQGTLVTVSS

SEQ ID NO: 11 - protein, 116 aa, Artificial Sequence
  Humanized 5H10 Heavy chain variable region VH4
QVQLVQSGAEVKKPGSSVKVSCKSSGYAFSSYWMNWVRQRPGQGLEWIGQIYPGDGDTHYNGKFKGRVTITADKSTSTAYMELSSLRSEDTAVYFCSSSNWVGSYWGQGTLVTVSS

SEQ ID NO: 12 - protein, 116 aa, Artificial Sequence
  Humanized 5H10 Heavy chain variable region VH5
QVQLVQSGAEVKKPGSSVKVSCKSSGYAFSSYWMNWVRQRPGQGLEWIGQIYPGDGDTHYNGKFQGRVTITADKSTSTAYMELSSLRSEDTAVYYCSSSNWVGSYWGQGTLVTVSS

SEQ ID NO: 13 - protein, 112 aa, Mus musculus
DVVMTQTPLTLSVTIGQTASISCKSSQSLLESDGKTYLNWLSQRPGQSPKRLIYLVSRLDSGVPDRFTGSGSGTDFTLKISRVEAEDLGVYYCWQGTHLPQTFGGGTKLEIK

SEQ ID NO: 14 - protein, 112 aa, Artificial Sequence
  Humanized 5H10 Light chain variable region VK1
DVVMTQSPLTLSVTLGQPASISCKSSQSLLESDGKTYLNWLQQRPGQSPRRLIYLVSRLDSGVPDRFTGSGSGTDFTLKISRVEAEDVGVYYCWQGTHLPQTFGGGTKVEIK

SEQ ID NO: 15 - protein, 112 aa, Artificial Sequence
  Humanized 5H10 Light chain variable region VK2
DVVMTQSPLSLPVTLGQPASISCKSSQSLLESDGKTYLNWLQQRPGQSPRRLIYLVSRLDSGVPDRFTGSGSGTDFTLKISRVEAEDVGVYYCWQGTHLPQTFGGGTKVEIK

SEQ ID NO: 16 - protein, 112 aa, Artificial Sequence
  Humanized 5H10 Light chain variable region VK3
DVVMTQSPLSLPVTLGQPASISCKSSQSLLESDGKTYLNWLQQRPGQSPRRLIYLVSRLDSGVPDRFSGSGSGTDFTLKISRVEAEDVGVYYCWQGTHLPQTFGGGTKVEIK

SEQ ID NO: 17 - protein, 112 aa, Artificial Sequence
  Humanized 5H10 Light chain variable region VK4
DVVMTQSPLSLPVTLGQPASISCKSSQSLLESDGKTYLNWFQQRPGQSPRRLIYLVSRLDSGVPDRFSGSGSGTDFTLKISRVEAEDVGVYYCWQGTHLPQTFGGGTKVEIK

SEQ ID NO: 18 - DNA, 348 bp, Mus musculus
caggttcagctgcagcagtctggggctgagctcgtgaggcctgggtcctcagtgaagatttcctgcaagtcttctggctatgcattcagtagctactggatgaactgggtgaagcagaggcctggacagggtcttgagtggattggacagatttatcctggagatggtgatactcactacaatggaaagttcaagggcaaagccacactgactgcagacaaatcctccagcacagcctacatgcagctcagcaggctaacatctgaggactctgcggtctatttctgttcaagttcaaactgggtcgggagttactggggccaagggactctggtcaccgtctcctca

SEQ ID NO: 19 - DNA, 348 bp, Artificial Sequence
  Humanized heavy chain variable region VH1
caggtccagctggtgcaatctggggctgagctgaagaagcctgggtcctcggtgaagatttcctgcaagtcttctggatatgcattcagcagctattggatgaactgggtgaagcagaggcctggacaagggcttgagtggattggacagatctatcctggagatggtgatactcactacaatggaaagttcaagggcaaagccacgctgaccgcggacaaatccacgagcacagcctacatggagctgagcagcctgacatctgaggactctgccgtgtatttctgttcaagttcaaactgggtcgggagttactggggccaaggaaccctggtcaccgtctcctca

SEQ ID NO: 20 - DNA, 348 bp, Artificial Sequence
  Humanized heavy chain variable region VH2
caggtccagctggtgcaatctggggctgaggtgaagaagcctgggtcctcggtgaagatttcctgcaagtcttctggatatgcattcagcagctattggatgaactgggtgaagcagaggcctggacaagggcttgagtggattggacagatctatcctggagatggtgatactcactacaatggaaagttcaagggcaaagccacgctgaccgcggacaaatccacgagcacagcctacatggagctgagcagcctgagatctgaggacacggccgtgtatttctgttcaagttcaaactgggtcgggagttactggggccaaggaaccctggtcaccgtctcctca

SEQ ID NO: 21 - DNA, 348 bp, Artificial Sequence
  Humanized heavy chain variable region VH3
caggtccagctggtgcaatctggggctgaggtgaagaagcctgggtcctcggtgaaggtttcctgcaagtcttctggatatgcattcagcagctattggatgaactgggtgcgacagaggcctggacaagggcttgagtggattggacagatctatcctggagatggtgatactcactacaatggaaagttcaagggcaaagccacgctgaccgcggacaaatccacgagcacagcctacatggagctgagcagcctgagatctgaggacacggccgtgtatttctgttcaagttcaaactgggtcgggagttactggggccaaggaaccctggtcaccgtctcctca

SEQ ID NO: 22 - DNA, 348 bp, Artificial Sequence
  Humanized heavy chain variable region VH4
caggtccagctggtgcaatctggggctgaggtgaagaagcctgggtcctcggtgaaggtttcctgcaagtcttctggatatgcattcagcagctattggatgaactgggtgcgacagaggcctggacaagggcttgagtggattggacagatctatcctggagatggtgatactcactacaatggaaagttcaagggcagagtcacgattaccgcggacaaatccacgagcacagcctacatggagctgagcagcctgagatctgaggacacggccgtgtatttctgttcaagttcaaactgggtcgggagttactggggccaaggaaccctggtcaccgtctcctca

SEQ ID NO: 23 - DNA, 348 bp, Artificial Sequence
  Humanized heavy chain variable region VH5
caggtccagctggtgcaatctggggctgaggtgaagaagcctgggtcctcggtgaaggtttcctgcaagtcttctggatatgcattcagcagctattggatgaactgggtgcgacagaggcctggacaagggcttgagtggattggacagatctatcctggagatggtgatactcactacaatggaaagttccagggcagagtcacgattaccgcggacaaatccacgagcacagcctacatggagctgagcagcctgagatctgaggacacggccgtgtattactgttcaagttcaaactgggtcgggagttactggggccaaggaaccctggtcaccgtctcctca

SEQ ID NO: 24 - DNA, 336 bp, Mus musculus
gatgttgtgatgacccagactccactcactttgtcggttaccattggacaaacagcctccatctcttgcaagtcaagtcagagcctcttagaaagtgatggaaagacatatttgaattggttgtcacagaggccaggccagtctccaaagcgcctaatctatctggtgtctagactggactctggagtccctgacaggttcactggcagtggatcagggacagatttcacactgaaaatcagcagagtggaggctgaggatttgggagtttattattgttggcaaggcacacatcttcctcagacgttcggtggaggcaccaagctggagatcaaa

SEQ ID NO: 25 - DNA, 336 bp, Artificial Sequence
  Humanized light chain variable region VK1
gatgttgtgatgactcagtctccactcactctgtcggtcacccttggacagccggcctccatctcctgcaagtctagtcaaagcctcttagaaagtgatggaaagacctacttgaattggttgcagcagaggccaggccaatctccaaggcgcctaatttatctggtttctagactggactctggggtcccagacagattcactggcagtgggtcaggcactgatttcacactgaaaatcagcagggtggaggctgaggatgttggggtttattactgctggcaaggcacacatcttcctcagactttcggcggagggaccaaggtggagatcaaa

SEQ ID NO: 26 - DNA, 336 bp, Artificial Sequence
  Humanized light chain variable region VK2
gatgttgtgatgactcagtctccactctccctgcccgtcacccttggacagccggcctccatctcctgcaagtctagtcaaagcctcttagaaagtgatggaaagacctacttgaattggttgcagcagaggccaggccaatctccaaggcgcctaatttatctggtttctagactggactctggggtcccagacagattcactggcagtgggtcaggcactgatttcacactgaaaatcagcagggtggaggctgaggatgttggggtttattactgctggcaaggcacacatcttcctcagactttcggcggagggaccaaggtggagatcaaa

SEQ ID NO: 27 - DNA, 336 bp, Artificial Sequence
  Humanized light chain variable region VK3
gatgttgtgatgactcagtctccactctccctgcccgtcacccttggacagccggcctccatctcctgcaagtctagtcaaagcctcttagaaagtgatggaaagacctacttgaattggttgcagcagaggccaggccaatctccaaggcgcctaatttatctggtttctagactggactctggggtcccagacagattcagcggcagtgggtcaggcactgatttcacactgaaaatcagcagggtggaggctgaggatgttggggtttattactgctggcaaggcacacatcttcctcagactttcggcggagggaccaaggtggagatcaaa

SEQ ID NO: 28 - DNA, 336 bp, Artificial Sequence
  Humanized light chain variable region VK4
gatgttgtgatgactcagtctccactctccctgcccgtcacccttggacagccggcctccatctcctgcaagtctagtcaaagcctcttagaaagtgatggaaagacctacttgaattggtttcagcagaggccaggccaatctccaaggcgcctaatttatctggtttctagactggactctggggtcccagacagattcagcggcagtgggtcaggcactgatttcacactgaaaatcagcagggtggaggctgaggatgttggggtttattactgctggcaaggcacacatcttcctcagactttcggcggagggaccaaggtggagatcaaa

SEQ ID NO: 29 - protein, 40 aa, Homo sapiens
PEKDSRVSVTKPFMLPPVAASSLRNDSSSSNRKAKNPPGD

SEQ ID NO: 30 - protein, 21 aa, Homo sapiens
ASSLRNDSSSSNRKAKNPPGD

SEQ ID NO: 31 - protein, 8 aa, Homo sapiens
SSNRKAKN

SEQ ID NO: 32 - protein, 14 aa, Homo sapiens
SSSSNRKAKNPPGD

SEQ ID NO: 33 - protein, 14 aa, Homo sapiens
ASSLRNDSSSSNRK

SEQ ID NO: 34 - protein, 29 aa, Homo sapiens
DSRVSVTKPFMLPPVAASSLRNDSSSSNR

SEQ ID NO: 35 - protein, 7 aa, Homo sapiens
SNRKAKN

SEQ ID NO: 36 - protein, 13 aa, Homo sapiens
ASSLRNDSSSSNR

SEQ ID NO: 37 - protein, 17 aa, Artificial Sequence
  VH5 CDR2
QIYPGDGDTHYNGKFQG

SEQ ID NO: 38 - protein, 443 aa, Artificial Sequence
  VH0 IgG4 heavy chain
QVQLQQSGAELVRPGSSVKISCKSSGYAFSSYWMNWVKQRPGQGLEWIGQIYPGDGDTHYNGKFKGKATLTADKSSSTAYMQLSRLTSEDSAVYFCSSSNWVGSYWGQGTLVTVSSASTKGPSVFPLAPCSRSTSESTAALGCLVKDYFPEPVTVSWNSGALTSGVHTFPAVLQSSGLYSLSSVVTVPSSSLGTKTYTCNVDHKPSNTKVDKRVESKYGPPCPPCPAPEFEGGPSVFLFPPKPKDTLMISRTPEVTCVVVDVSQEDPEVQFNWYVDGVEVHNAKTKPREEQFNSTYRVVSVLTVLHQDWLNGKEYKCKVSNKGLPSSIEKTISKAKGQPREPQVYTLPPSQEEMTKNQVSLTCLVKGFYPSDIAVEWESNGQPENNYKTTPPVLDSDGSFFLYSRLTVDKSRWQEGNVFSCSVMHEALHNHYTQKSLSLSLGK

SEQ ID NO: 39 - protein, 219 aa, Artificial Sequence
  VK0 Kappa light chain
DVVMTQTPLTLSVTIGQTASISCKSSQSLLESDGKTYLNWLSQRPGQSPKRLIYLVSRLDSGVPDRFTGSGSGTDFTLKISRVEAEDLGVYYCWQGTHLPQTFGGGTKLEIKRTVAAPSVFIFPPSDEQLKSGTASVVCLLNNFYPREAKVQWKVDNALQSGNSQESVTEQDSKDSTYSLSSTLTLSKADYEKHKVYACEVTHQGLSSPVTKSFNRGEC

SEQ ID NO: 40 - protein, 327 aa, Artificial Sequence
  heavy chain constant region
ASTKGPSVFPLAPCSRSTSESTAALGCLVKDYFPEPVTVSWNSGALTSGVHTFPAVLQSSGLYSLSSVVTVPSSSLGTKTYTCNVDHKPSNTKVDKRVESKYGPPCPPCPAPEFEGGPSVFLFPPKPKDTLMISRTPEVTCVVVDVSQEDPEVQFNWYVDGVEVHNAKTKPREEQFNSTYRVVSVLTVLHQDWLNGKEYKCKVSNKGLPSSIEKTISKAKGQPREPQVYTLPPSQEEMTKNQVSLTCLVKGFYPSDIAVEWESNGQPENNYKTTPPVLDSDGSFFLYSRLTVDKSRWQEGNVFSCSVMHEALHNHYTQKSLSLSLGK

SEQ ID NO: 41 - protein, 107 aa, Homo sapiens [sequence omitted]

SEQ ID NO: 42 - protein, 443 aa, Artificial Sequence
  5H10 VH1 Heavy Chain
QVQLVQSGAELKKPGSSVKISCKSSGYAFSSYWMNWVKQRPGQGLEWIGQIYPGDGDTHYNGKFKGKATLTADKSTSTAYMELSSLTSEDSAVYFCSSSNWVGSYWGQGTLVTVSSASTKGPSVFPLAPCSRSTSESTAALGCLVKDYFPEPVTVSWNSGALTSGVHTFPAVLQSSGLYSLSSVVTVPSSSLGTKTYTCNVDHKPSNTKVDKRVESKYGPPCPPCPAPEFEGGPSVFLFPPKPKDTLMISRTPEVTCVVVDVSQEDPEVQFNWYVDGVEVHNAKTKPREEQFNSTYRVVSVLTVLHQDWLNGKEYKCKVSNKGLPSSIEKTISKAKGQPREPQVYTLPPSQEEMTKNQVSLTCLVKGFYPSDIAVEWESNGQPENNYKTTPPVLDSDGSFFLYSRLTVDKSRWQEGNVFSCSVMHEALHNHYTQKSLSLSLGK

SEQ ID NO: 43 - protein, 443 aa, Artificial Sequence
  5H10 VH2 Heavy Chain
QVQLVQSGAEVKKPGSSVKISCKSSGYAFSSYWMNWVKQRPGQGLEWIGQIYPGDGDTHYNGKFKGKATLTADKSTSTAYMELSSLRSEDTAVYFCSSSNWVGSYWGQGTLVTVSSASTKGPSVFPLAPCSRSTSESTAALGCLVKDYFPEPVTVSWNSGALTSGVHTFPAVLQSSGLYSLSSVVTVPSSSLGTKTYTCNVDHKPSNTKVDKRVESKYGPPCPPCPAPEFEGGPSVFLFPPKPKDTLMISRTPEVTCVVVDVSQEDPEVQFNWYVDGVEVHNAKTKPREEQFNSTYRVVSVLTVLHQDWLNGKEYKCKVSNKGLPSSIEKTISKAKGQPREPQVYTLPPSQEEMTKNQVSLTCLVKGFYPSDIAVEWESNGQPENNYKTTPPVLDSDGSFFLYSRLTVDKSRWQEGNVFSCSVMHEALHNHYTQKSLSLSLGK

SEQ ID NO: 44 - protein, 443 aa, Artificial Sequence
  5H10 VH3 Heavy Chain
QVQLVQSGAEVKKPGSSVKVSCKSSGYAFSSYWMNWVRQRPGQGLEWIGQIYPGDGDTHYNGKFKGKATLTADKSTSTAYMELSSLRSEDTAVYFCSSSNWVGSYWGQGTLVTVSSASTKGPSVFPLAPCSRSTSESTAALGCLVKDYFPEPVTVSWNSGALTSGVHTFPAVLQSSGLYSLSSVVTVPSSSLGTKTYTCNVDHKPSNTKVDKRVESKYGPPCPPCPAPEFEGGPSVFLFPPKPKDTLMISRTPEVTCVVVDVSQEDPEVQFNWYVDGVEVHNAKTKPREEQFNSTYRVVSVLTVLHQDWLNGKEYKCKVSNKGLPSSIEKTISKAKGQPREPQVYTLPPSQEEMTKNQVSLTCLVKGFYPSDIAVEWESNGQPENNYKTTPPVLDSDGSFFLYSRLTVDKSRWQEGNVFSCSVMHEALHNHYTQKSLSLSLGK

SEQ ID NO: 45 - protein, 443 aa, Artificial Sequence
  5H10 VH4 Heavy Chain
QVQLVQSGAEVKKPGSSVKVSCKSSGYAFSSYWMNWVRQRPGQGLEWIGQIYPGDGDTHYNGKFKGRVTITADKSTSTAYMELSSLRSEDTAVYFCSSSNWVGSYWGQGTLVTVSSASTKGPSVFPLAPCSRSTSESTAALGCLVKDYFPEPVTVSWNSGALTSGVHTFPAVLQSSGLYSLSSVVTVPSSSLGTKTYTCNVDHKPSNTKVDKRVESKYGPPCPPCPAPEFEGGPSVFLFPPKPKDTLMISRTPEVTCVVVDVSQEDPEVQFNWYVDGVEVHNAKTKPREEQFNSTYRVVSVLTVLHQDWLNGKEYKCKVSNKGLPSSIEKTISKAKGQPREPQVYTLPPSQEEMTKNQVSLTCLVKGFYPSDIAVEWESNGQPENNYKTTPPVLDSDGSFFLYSRLTVDKSRWQEGNVFSCSVMHEALHNHYTQKSLSLSLGK

SEQ ID NO: 46 - protein, 443 aa, Artificial Sequence
  5H10 VH5 Heavy Chain
QVQLVQSGAEVKKPGSSVKVSCKSSGYAFSSYWMNWVRQRPGQGLEWIGQIYPGDGDTHYNGKFQGRVTITADKSTSTAYMELSSLRSEDTAVYYCSSSNWVGSYWGQGTLVTVSSASTKGPSVFPLAPCSRSTSESTAALGCLVKDYFPEPVTVSWNSGALTSGVHTFPAVLQSSGLYSLSSVVTVPSSSLGTKTYTCNVDHKPSNTKVDKRVESKYGPPCPPCPAPEFEGGPSVFLFPPKPKDTLMISRTPEVTCVVVDVSQEDPEVQFNWYVDGVEVHNAKTKPREEQFNSTYRVVSVLTVLHQDWLNGKEYKCKVSNKGLPSSIEKTISKAKGQPREPQVYTLPPSQEEMTKNQVSLTCLVKGFYPSDIAVEWESNGQPENNYKTTPPVLDSDGSFFLYSRLTVDKSRWQEGNVFSCSVMHEALHNHYTQKSLSLSLGK

SEQ ID NO: 47 - protein, 219 aa, Artificial Sequence
  5H10 VK1 Light Chain
DVVMTQSPLTLSVTLGQPASISCKSSQSLLESDGKTYLNWLQQRPGQSPRRLIYLVSRLDSGVPDRFTGSGSGTDFTLKISRVEAEDVGVYYCWQGTHLPQTFGGGTKVEIKRTVAAPSVFIFPPSDEQLKSGTASVVCLLNNFYPREAKVQWKVDNALQSGNSQESVTEQDSKDSTYSLSSTLTLSKADYEKHKVYACEVTHQGLSSPVTKSFNRGEC

SEQ ID NO: 48 - protein, 219 aa, Artificial Sequence
  5H10 VK2 Light Chain
DVVMTQSPLSLPVTLGQPASISCKSSQSLLESDGKTYLNWLQQRPGQSPRRLIYLVSRLDSGVPDRFTGSGSGTDFTLKISRVEAEDVGVYYCWQGTHLPQTFGGGTKVEIKRTVAAPSVFIFPPSDEQLKSGTASVVCLLNNFYPREAKVQWKVDNALQSGNSQESVTEQDSKDSTYSLSSTLTLSKADYEKHKVYACEVTHQGLSSPVTKSFNRGEC

SEQ ID NO: 49 - protein, 219 aa, Artificial Sequence
  5H10 VK3 Light Chain
DVVMTQSPLSLPVTLGQPASISCKSSQSLLESDGKTYLNWLQQRPGQSPRRLIYLVSRLDSGVPDRFSGSGSGTDFTLKISRVEAEDVGVYYCWQGTHLPQTFGGGTKVEIKRTVAAPSVFIFPPSDEQLKSGTASVVCLLNNFYPREAKVQWKVDNALQSGNSQESVTEQDSKDSTYSLSSTLTLSKADYEKHKVYACEVTHQGLSSPVTKSFNRGEC

SEQ ID NO: 50 - protein, 219 aa, Artificial Sequence
  5H10 VK4 Light Chain
DVVMTQSPLSLPVTLGQPASISCKSSQSLLESDGKTYLNWFQQRPGQSPRRLIYLVSRLDSGVPDRFSGSGSGTDFTLKISRVEAEDVGVYYCWQGTHLPQTFGGGTKVEIKRTVAAPSVFIFPPSDEQLKSGTASVVCLLNNFYPREAKVQWKVDNALQSGNSQESVTEQDSKDSTYSLSSTLTLSKADYEKHKVYACEVTHQGLSSPVTKSFNRGEC